European Patent Application EP 4 650 453 A1, published November 19, 2025. Title: ANTIBIOTIC-FREE MINIPLASMID, AND PREPARATION METHOD THEREFOR AND USE THEREOF. Applicant: Maxirna (Shanghai) Pharmaceutical Co., Ltd. The sequence listing filed with the application follows.

SEQUENCE LISTING (47 sequences)

SEQ ID NO: 1 - protein, 50 aa, synthetic construct
MSTDERKLEIIRKVSSDIDEPTLEAIEYLLSTPSDIPEPILRVIEQAMAE

SEQ ID NO: 2 - protein, 60 aa, synthetic construct
MSTDERKLEIIRKVSSDIDEPTLEAIEYLLSTPSDIPEPILRVIEQAMAEEPLEEYTSAK

SEQ ID NO: 3 - protein, 68 aa, synthetic construct
MSTDERKLEIIRKVSSDIDEPTLEAIEYLLSTPSDIPEPILRVIEQAMAEEPLEEYTSAKEVIEKSRT

SEQ ID NO: 4 - protein, 102 aa, synthetic construct
MKVRWTHTAKKSLNQVYEFLNDVWGNRVADHFLQLVDAKINSLAKRPEIGKKHFNRDFRSILIHKHVRLFYRVGNSEIVLLTFWDNRQDPVRLAESLTKKKP

SEQ ID NO: 5 - DNA, 207 bp, synthetic construct
  source 1..207: mol_type = other DNA
atgtcaacagacgaaagaaaattggagataatcagaaaagtgagttctgatatagacgagcctactctcgaagcaattgaatatttgttatcaaccccttcggatatcccagaacctatactgagagttatagaacaagcaatggcagaagaacctttagaggaatatacttcagctaaagaggttattgagaaaagccgaacctaa

SEQ ID NO: 6 - DNA, 309 bp, synthetic construct
  source 1..309: mol_type = other DNA
atgaaggtcagatggacacacactgcgaaaaaatctctcaaccaagtttatgaatttttaaatgacgtttggggaaaccgtgtagccgaccattttttacagttggtagatgcaaaaatcaattctctggccaaaaggcctgagattggtaaaaagcactttaaccgtgattttagatcaatactaattcacaaacatgttcggcttttttaccgtgttggaaattcagaaatagttcttctcaccttttgggacaatcgacaggatcctgtcagacttgcagaatctctgacaaaaaagaagccctaa

SEQ ID NO: 7 - DNA, 207 bp, synthetic construct
  source 1..207: mol_type = other DNA
atgtcaacagatgaaagaaaattggagatcatcagaaaagtgagttctgatattgatgagcctactctggaagcaattgaatatttgttatcaaccccttcagatatcccagaaccaatactgagagttattgaacaagcaatggcagaagaacctcttgaggaatacacttcagccaaagaggttattgagaaaagcagaacctaa

SEQ ID NO: 8 - DNA, 559 bp, synthetic construct
  source 1..559: mol_type = other DNA
gaattcttaattaaaatcagcagttcaacctgttgatagtatgtactaagctctcatgtttaatgtactaagctctcatgtttaatgaactaaaccctcatggctaatgtactaagctctcatggctaatgtactaagctctcatgtttcatgtactaagctctcatgtttgaacaataaaattaatataaatcagcaacttaaatagcctctaaggttttaagttttataagaaaaaaaagaatatataaggcttttaaaggttttaaggtttcctagctttaggttctgcttttctcaataacctctttggctgaagtgtattcctcaagaggttcttctgccattgcttgttcaataactctcagtattggttctgggatatctgaaggggttgataacaaatattcaattgcttccagagtaggctcatcaatatcagaactcacttttctgatgatctccaattttctttcatctgttgacatgatggccctcctatagtgagttgtattatactatgcagatatactatgccaatgtttaattgtcaactagt

SEQ ID NO: 9 - protein, 69 aa, synthetic construct
MPKKATNLSLNSELLAEAKRLNINLSATMEKALEKEVRQRLKTEWLKQNAEGINACNELTENHGLFSDS

SEQ ID NO: 10 - protein, 73 aa, synthetic construct
MPKKATNLSLNSELLAEAKRLNINLSATMEKALEKEVRQRLKTEWLKQNAEGINACNELTENHGLFSDSYRVF

SEQ ID NO: 11 - protein, 77 aa, synthetic construct
MRNAYSTQAPKKATNLSLNSELLAEAKRLNINLSATMEKALEKEVRQRLKTEWLKQNAEGINACNELTENHGLFSDS

SEQ ID NO: 12 - protein, 81 aa, synthetic construct
MRNAYSTQAPKKATNLSLNSELLAEAKRLNINLSATMEKALEKEVRQRLKTEWLKQNAEGINACNELTENHGLFSDSYRVF

SEQ ID NO: 13 - protein, 105 aa, synthetic construct
MSQFSLYKNNDKNTATAYPYFVDVQSGLLDTLNTRLVIPLTPTELLEKKAPSHLCPVIHIDEGDFVILTHQMASVPTKILREPVSNLSTFRDEIISAIDFLITGI

SEQ ID NO: 14 - DNA, 246 bp, synthetic construct
  source 1..246: mol_type = other DNA
atgagaaatgcatatagtacgcaagcaccaaagaaagctacaaacttaagcttaaacagtgagttacttgcggaggctaaacggttaaatataaacctttcggcaacaatggaaaaggcacttgaaaaagaagtacgtcaacgccttaagactgaatggttaaagcaaaatgctgagggcattaatgcttgtaacgagctaactgaaaatcatggactattttctgattcttaccgagtattctaa

SEQ ID NO: 15 - DNA, 318 bp, synthetic construct
  source 1..318: mol_type = other DNA
atgtcacaattctcgctatacaaaaacaacgataaaaacacagcaaccgcatacccatactttgttgacgttcaaagtggattgctggatacattgaacactcggttagttattccgttgacgcctactgagttgttagagaaaaaagcacctagtcatctatgtcccgtaatccatattgatgaaggtgacttcgtaattctgacgcatcaaatggcaagtgtaccaaccaaaattctaagagagcctgtaagcaatctaagcacttttagagacgagatcatctctgctatcgattttcttattacgggcatataa

SEQ ID NO: 16 - DNA, 246 bp, synthetic construct
  source 1..246: mol_type = other DNA
atgagaaatgcatatagtacccaagcaccaaagaaagctacaaacctgagcttaaacagtgagttacttgcagaggctaaaagattaaatataaaccttagtgcaacaatggaaaaggcacttgaaaaagaagtaagacaaagactgaagactgaatggttaaagcaaaatgctgagggcattaatgcttgtaatgagctaactgaaaatcatggactattttctgattcttacagagtattctaa

SEQ ID NO: 17 - DNA, 592 bp, synthetic construct
  source 1..592: mol_type = other DNA
ttaattaaaatcagcagttcaacctgttgatagtatgtactaagctctcatgtttaatgtactaagctctcatgtttaatgaactaaaccctcatggctaatgtactaagctctcatggctaatgtactaagctctcatgtttcatgtactaagctctcatgtttgaacaataaaattaatataaatcagcaacttaaatagcctctaaggttttaagttttataagaaaaaaaagaatatataaggcttttaaaggttttaaggtttcctagctttagaatactctgtaagaatcagaaaatagtccatgattttcagttagctcattacaagcattaatgccctcagcattttgctttaaccattcagtcttcagtctttgtcttacttctttttcaagtgccttttccattgttgcactaaggtttatatttaatcttttagcctctgcaagtaactcactgtttaagctcaggtttgtagctttctttggtgcttgggtactatatgcatttctcatgatggccctcctatagtgagttgtattatactatgcagatatactatgccaatgtttaattgtcaactagt

SEQ ID NO: 18 - DNA, 631 bp, synthetic construct
  source 1..631: mol_type = other DNA
ttaattaaaatcagcagttcaacctgttgatagtatgtactaagctctcatgtttaatgtactaagctctcatgtttaatgaactaaaccctcatggctaatgtactaagctctcatggctaatgtactaagctctcatgtttcatgtactaagctctcatgtttgaacaataaaattaatataaatcagcaacttaaatagcctctaaggttttaagttttataagaaaaaaaagaatatataaggcttttaaaggttttaaggtttcctagctctatttgtggcatgtaggggctgcctgttcattttcacttccccaggactccagccaactcaccacttcatcacctgtgacatgcaagcctgatgtctggtgttcttcccatgctcttaatgcttcttgctgcaaagcttctcttttctcttctctctcaacatattctctgattgcttctctcatcatccagtgtgatgatctttttctggtttctgctaaatgctccactctggctttaatatctgcatctaatttaactgacactggtttgattgtgctcatgatggccctcctatagtgagttgtattatactatgcagatatactatgccaatgtttaattgtcaactagt

SEQ ID NO: 19 - DNA, 571 bp, synthetic construct
  source 1..571: mol_type = other DNA
gaattcttaattaaaatcagcagttcaacctgttgatagtatgtactaagctctcatgtttaatgtactaagctctcatgtttaatgaactaaaccctcatggctaatgtactaagctctcatggctaatgtactaagctctcatgtttcatgtactaagctctcatgtttgaacaataaaattaatataaatcagcaacttaaatagcctctaaggttttaagttttataagaaaaaaaagaatatataaggcttttaaaggttttaaggtttcctagcttcaccagtccctgttctcatcagcaaaagagccattcatttcaataaatctggccacctcagccatcccttcctgattttctgctttccatctttctgctctcagtcttctggcttcattctgcatggttgtgcttaccagacctgagatattgacatcatatgccttgagcaactgatagctgtcactgtcaactgtcactgtaattctctgcttcatgatggccctcctatagtgagttgtattatactatgcagatatactatgccaatgtttaattgtcaactagt

SEQ ID NO: 20 - DNA, 267 bp, synthetic construct
  source 1..267: mol_type = other DNA
aatcagcagttcaacctgttgatagtatgtactaagctctcatgtttaatgtactaagctctcatgtttaatgaactaaaccctcatggctaatgtactaagctctcatggctaatgtactaagctctcatgtttcatgtactaagctctcatgtttgaacaataaaattaatataaatcagcaacttaaatagcctctaaggttttaagttttataagaaaaaaaagaatatataaggcttttaaaggttttaaggtttcctagct

SEQ ID NO: 21 - protein, 102 aa, synthetic construct
MSTIKPVSVKLDADIKARVEHLAETRKRSSHWMMREAIREYVEREEKREALQQEALRAWEEHQTSGLHVTGDEVVSWLESWGSENEQAALHATNSLHCHCIT

SEQ ID NO: 22 - protein, 97 aa, synthetic construct
MPQIVFTATALRDLERLREFLRSKNPPAAQRAASAIINTIRKLESYPDIGRPIDDNDFSFRELLIDFGDTGYLAMYQYDGGERLTVLCIRHQKEAGY

SEQ ID NO: 23 - DNA, 285 bp, synthetic construct
  source 1..285: mol_type = other DNA
atgagcacaatcaaacccgtgtcggttaaattagatgccgatattaaagccagagtcgagcatttagcggaaacccgtaaacgttcatcacactggatgatgcgtgaagcgatccgtgaatatgttgagagagaagagaaacgcgaagctttgcagcaagaagcgttacgcgcatgggaagaacaccagacatcaggcttgcatgtcaccggtgacgaagtggtgagttggctggagtcctggggaagtgaaaatgaacaggcagcccctacatgccacaaatag

SEQ ID NO: 24 - DNA, 294 bp, synthetic construct
  source 1..294: mol_type = other DNA
atgccacaaatagtcttcactgccactgcattacgtgatttagaacgcttacgtgagtttcttcgcagtaaaaatccccctgccgcacaacgggctgccagcgccataatcaataccattagaaaactggaaagctatccagacattggtcggcctatcgatgacaatgactttagctttagggaactgctcatcgactttggtgacacgggctatctggcaatgtaccagtatgatggcggcgaacgattgaccgtgttgtgtatccgccaccaaaaagaagccggatattga

SEQ ID NO: 25 - DNA, 231 bp, synthetic construct
  source 1..231: mol_type = other DNA
atgagaaccgtatccatttttaaaaatggcaacaaccgtgctatccgccttccacgcgatctggattttgagggggtgagcgagctggagatcgtccgggaaggggacagcatcattctgcgccccgtccggccgacctggggctcattcctggagctagaaaaggccgatccggactttatgacggagcgcgaggacgttgtcagcgacgaaggacgagttaacctgtga

SEQ ID NO: 26 - DNA, 417 bp, synthetic construct
  source 1..417: mol_type = other DNA
gtgaacaagatctatatgctcgacacgaacatctgctcgttcatcatgcgcgagcaacctgaagcattgcttaagcacctggagcagtcggtgctgcgcggtcaccgtatcgtggtctcggccatcacctactccgagatgcgcttcggtgccaccggtccgaaggcctcgccacgccacgtgcaactggttgacgcgttctgtgagaggctcgatgccgtcctgccgtgggaccgcgccgcggtggatgcgaccacggagattaaggtggcactgcgtctcgccggcacgccgatcggtccgaacgacacggcgatagccggacacgccatcgctgcctgtgccattctggtgacgaataatgtgagagagtttgagcgggtaccgggtcttgtgctggaagactgggtaagataa

SEQ ID NO: 27 - protein, 86 aa, synthetic construct
MSSRTMTVDTGEELRAFVEGLVESGDYKTNSEVIRDGLRLLQEKTAGSKLAALRQLIDEGEQSGEAVPWDRDSFLARMRQKGPRGG

SEQ ID NO: 28 - protein, 98 aa, synthetic construct
MVANTLVLKPRAEQDLERIFEYSYTEFGWQQAQQYISDLDQTFQTLAASTDLAINYDHVRPGLKAFPVGAHIVFFRATDTGIEVIRVLHQSMDYPRHV

SEQ ID NO: 29 - protein, 261 aa, synthetic construct
ATGTCATCTCGAACTATGACGGTTGATACCGGTGAAGAATTGCGCGCCTTTGTTGAAGGCCTGGTGGAATCTGGCGACTATAAGACCAACAGCGAAGTGATCCGCGATGGGCTCCGTCTGCTGCAGGAAAAAACCGCCGGGTCTAAACTGGCAGCATTGCGCCAGCTCATTGATGAAGGTGAGCAAAGTGGCGAAGCTGTGCCCTGGGATCGAGATAGCTTTTTAGCCCGCATGAGGCAAAAAGGCCCGCGTGGTGGCTAA

SEQ ID NO: 30 - DNA, 294 bp, synthetic construct
  source 1..294: mol_type = other DNA
gtggctaatactctggtcctcaaaccccgtgcggaacaagatttagaacgcatttttgaatacagctatacggagtttggctggcaacaggcgcagcagtatatcagcgatctggaccagacctttcagacactcgcggcatcgaccgatctggctattaattacgatcatgtccgtcccggcctgaaagcctttccggtcggcgcccatatcgtattcttccgcgccacagacaccggcatcgaagtgatccgggtgctgcatcaatccatggactacccacgtcatgtgtga

SEQ ID NO: 31 - DNA, 291 bp, synthetic construct
  source 1..291: mol_type = other DNA
atgcgaccgtctgttgtgcttgacatgaagcgaagcgcagtgcgtgaagcggtaggccgctttcgcgccgcgaacccgcgcgtcttcggctcggtgctgcatggcaccgaccgggatggcagcgacctcgacctgttggtcgatgcgctgcccggtgccacgttgttggacttgggcgatttggaagaagaactgaaatcgctgctcggcgttgacgtcgatctgctgactcccggcgacctgccgccgaagttccgggccaaggtgctcgcggaggcgcaaccgatatga

SEQ ID NO: 32 - DNA, 402 bp, synthetic construct
  source 1..402: mol_type = other DNA
atgagcgagaaccgcctgcccgattacctcgaccacattcagcaggccgcaaccgatgcgcgcagcttcgtggaagggatggccaaggacgacttcttggccgacaagcgcacccagcaggccgtcatcatgagcctgatcgtcatcggcgaggcggccacaaaggtgatggatggctacgtcgagttcacccaggcgcatgccgacgtgccgtggcgcagcatgcgcaatatgcgtaatcgcatggctcacggctatttcgacatcaacctcgatgtggtgtgggagacggtacaggaatggctgccggcgttgctccagcaattgcccgccgtgcgtcaggatgccgacgatgaagaccgtaacgacaactgtgaaagagggatctccgatgactgttga

SEQ ID NO: 33 - protein, 72 aa, synthetic construct
MKQRITVTVDSDSYQLLKAYDVNISGLVSTTMQNEARRLRAERWKAENQEGMAEVARFIEMNGSFADENRDW

SEQ ID NO: 34 - protein, 101 aa, synthetic construct
MQFKVYTYKRESRYRLFVDVQSDIIDTPGRRMVIPLASARLLSDKVSRELYPVVHIGDESWRMMTTDMASVPVSVIGEEVADLSHRENDIKNAINLMFWGI

SEQ ID NO: 35 - DNA, 219 bp, synthetic construct
  source 1..219: mol_type = other DNA
atgaagcagcgtattacagtgacagttgacagcgacagctatcagttgctcaaggcatatgatgtcaatatctccggtctggtaagcacaaccatgcagaatgaagcccgtcgtctgcgtgccgaacgctggaaagcggaaaatcaggaagggatggctgaggtcgcccggtttattgaaatgaacggctcttttgctgacgagaacagggactggtga

SEQ ID NO: 36 - DNA, 272 bp, synthetic construct
  source 1..272: mol_type = other DNA
gccgttatcgtctgtttgtggatgtacagagtgatattattgacacgcccgggcgacggatggtgatccccctggccagtgcacgtctgctgtcagataaagtctcccgtgaactttacccggtggtgcatatcggggatgaaagctggcgcatgatgaccaccgatatggccagtgtgccggtctccgttatcggggaagaagtggctgatctcagccaccgcgaaaatgacatcaaaaacgccattaacctgatgttctggggaatataa

SEQ ID NO: 37 - DNA, 285 bp, synthetic construct
  source 1..285: mol_type = other DNA
atgagcacaatcaaaccagtgtcagttaaattagatgcagatattaaagccagagtggagcatttagcagaaaccagaaaaagatcatcacactggatgatgagagaagcaatcagagaatatgttgagagagaagagaaaagagaagctttgcagcaagaagcattaagagcatgggaagaacaccagacatcaggcttgcatgtcacaggtgatgaagtggtgagttggctggagtcctggggaagtgaaaatgaacaggcagcccctacatgccacaaatag

SEQ ID NO: 38 - DNA, 219 bp, synthetic construct
  source 1..219: mol_type = other DNA
atgaagcagagaattacagtgacagttgacagtgacagctatcagttgctcaaggcatatgatgtcaatatctcaggtctggtaagcacaaccatgcagaatgaagccagaagactgagagcagaaagatggaaagcagaaaatcaggaagggatggctgaggtggccagatttattgaaatgaatggctcttttgctgatgagaacagggactggtga

SEQ ID NO: 39 - DNA, 291 bp, synthetic construct
  source 1..291: mol_type = other DNA
atgagaccatctgttgtgcttgacatgaagagaagtgcagtgagagaagcagtaggcagatttagagcagcaaacccaagagtctttggctcagtgctgcatggcacagacagagatggcagtgacctggacctgttggtggatgcactgccaggtgccaccttgttggacttgggagatttggaagaagaactgaaatcactgctgggagttgatgtggatctgctgactccaggagacctgccaccaaagttcagagccaaggtgctggcagaggcacaaccaatatga

SEQ ID NO: 40 - DNA, 231 bp, synthetic construct
  source 1..231: mol_type = other DNA
atgagaacagtatccatttttaaaaatggcaacaacagagctatcagacttccaagagatctggattttgagggggtgagtgagctggagattgtcagagaaggggacagcatcattctgagaccagtcagaccaacctggggctcattcctggagctagaaaaggcagatccagactttatgacagagagagaggatgttgtcagtgatgaaggaagagttaacctgtga

SEQ ID NO: 41 - DNA, 720 bp, synthetic construct
  source 1..720: mol_type = other DNA
atggtgagcaagggagaggagctgttcactggggtggtgcccatcctggtggagctggatggagatgtgaatggccacaagttctctgtgtctggagagggagagggagatgccacctatggcaagctgaccctgaagttcatctgcaccacaggcaagctgcctgtgccctggcccaccctggtgaccaccctgacctatggagtgcagtgcttcagcagataccctgaccacatgaagcagcatgacttcttcaagtctgccatgcctgagggctatgtccaggagagaaccatcttcttcaaggatgatggcaactacaagaccagagctgaggtgaagtttgagggagacaccctggtgaacagaattgagctgaagggcattgacttcaaggaggatggcaacatcctggggcacaagctggagtacaactacaacagccacaatgtctatatcatggctgacaagcagaagaatggcatcaaggtgaacttcaagatcagacacaacattgaggatggctctgtgcagctggctgaccactaccagcagaacacccccattggagatggccctgtgctgctgcctgacaaccactacctgagcacccagtctgccctgagcaaggaccccaatgagaagagagatcacatggtcctgctggagtttgtgacagctgctgggatcactctgggcatggatgagctgtacaagtaa

SEQ ID NO: 42 - protein, 239 aa, synthetic construct
MVSKGEELFTGVVPILVELDGDVNGHKFSVSGEGEGDATYGKLTLKFICTTGKLPVPWPTLVTTLTYGVQCFSRYPDHMKQHDFFKSAMPEGYVQERTIFFKDDGNYKTRAEVKFEGDTLVNRIELKGIDFKEDGNILGHKLEYNYNSHNVYIMADKQKNGIKVNFKIRHNIEDGSVQLADHYQQNTPIGDGPVLLPDNHYLSTQSALSKDPNEKRDHMVLLEFVTAAGITLGMDELYK

SEQ ID NO: 43 - protein, 40 aa, synthetic construct
MRNAYSTQAPKKATNLSLNSELLAEAKRLNINLSATMEKA

SEQ ID NO: 44 - protein, 29 aa, synthetic construct
MRNAYSTQAPKKATNLSLNSELLAEAKRL

SEQ ID NO: 45 - DNA, 2812 bp, synthetic construct
  source 1..2812: mol_type = other DNA
catggtgagcaagggcgaggagctgttcaccggggtggtgcccatcctggtcgagctggacggcgacgtaaacggccacaagttcagcgtgtccggcgagggcgagggcgatgccacctacggcaagctgaccctgaagttcatctgcaccaccggcaagctgcccgtgccctggcccaccctcgtgaccaccctgacctacggcgtgcagtgcttcagccgctaccccgaccacatgaagcagcacgacttcttcaagtccgccatgcccgaaggctacgtccaggagcgcaccatcttcttcaaggacgacggcaactacaagacccgcgccgaggtgaagttcgagggcgacaccctggtgaaccgcatcgagctgaagggcatcgacttcaaggaggacggcaacatcctggggcacaagctggagtacaactacaacagccacaacgtctatatcatggccgacaagcagaagaacggcatcaaggtgaacttcaagatccgccacaacatcgaggacggcagcgtgcagctcgccgaccactaccagcagaacacccccatcggcgacggccccgtgctgctgcccgacaaccactacctgagcacccagtccgccctgagcaaagaccccaacgagaagcgcgatcacatggtcctgctggagttcgtgaccgccgccgggatcactctcggcatggacgagctgtacaagtaaggatcctgcactagtgctgtcgactggtggactggtggactggtggactggtggactggtggactggtggactggtggactggtggactggtggactggtggacaagcttaaaaaaaaaaaaaaaaaaaaaaaaaaaaaaaaaaaaaaaaaaaaaaaaaaaaaaaaaaaaggaaaaaaaaaaaaaaaaaaaaaaaaaaaaaaaaaaaaaaaaaaaaaaaaaaaaaaaaaaaaggagaccgctagcacatgtgagcaaaaggccagcaaaaggccaggaaccgtaaaaaggccgcgttgctggcgtttttccataggctccgcccccctgacgagcatcacaaaaatcgacgctcaagtcagaggtggcgaaacccgacaggactataaagataccaggcgtttccccctggaagctccctcgtgcgctctcctgttccgaccctgccgcttaccggatacctgtccgcctttctcccttcgggaagcgtggcgctttctcatagctcacgctgtaggtatctcagttcggtgtaggtcgttcgctccaagctgggctgtgtgcacgaaccccccgttcagcccgaccgctgcgccttatccggtaactatcgtcttgagtccaacccggtaagacacgacttatcgccactggcagcagccactggtaacaggattagcagagcgaggtatgtaggcggtgctacagagttcttgaagtggtggcctaactacggctacactagaagaacagtatttggtatctgcgctctgctgaagccagttaccttcggaaaaagagttggtagctcttgatccggcaaacaaaccaccgctggtagcggtggtttttttgtttgcaagcagcagattacgcgcagaaaaaaaggatctcaagaagatcctttgatcttttctacggggtctgacgctcagtggaacgaaaactcacgttaagggattttggtcatgagattatcaaaaaggatcttcacctagatccttttaaattaaaaatgaagttttaaatcaatctaaagtatatatgagtaaacttggtctgacagttagaaaaactcatcgagcatcaaatgaaactgcaatttattcatatcaggattatcaataccatatttttgaaaaagccgtttctgtaatgaaggagaaaactcaccgaggcagttccataggatggcaagatcctggtatcggtctgcgattccgactcgtccaacatcaatacaacctattaatttcccctcgtcaaaaataaggttatcaagtgagaaatcaccatgagtgacgactgaatccggtgagaatggcaaaagtttatgcatttctttccagacttgttcaacaggccagccattacgctcgtcatcaaaatcactcgcatcaaccaaaccgttattcattcgtgattgcgcctgagcgagacgaaatacgcgatcgctgttaaaaggacaattacaaacaggaatcgaatgcaaccggcgcaggaacactgccagcgcatcaacaatattttcacctgaatcaggatattcttctaatacctggaatgctgttttcccagggatcgcagtggtgagtaaccatgcatcatcaggagtacggataaaatgcttgatggtcggaagaggcataaattccgtcagccagtttagtctgaccatctcatctgtaacatcattggcaacgctacctttgccatgtttcagaaacaactctggcgcatcgggcttcccatacaatcgatagattgtcgcacctgattgcccgacattatcgcgagcccatttatacccatataaatcagcatccatgttggaatttaatcgcggcctagagcaagacgtttcccgttgaatatggctcatactcttcctttttcaatattattgaagcatttatcagggttattgtctcatgagcggatacatatttgaatgtatttagaaaaataaacaaataggggttccgcgcacatttccccgaaaagtgccacctgacgtctaatacgactcactataagggaaataagagagaaaagaagagtaagaagaaatataagaccccggcgccgccac

SEQ ID NO: 46 - DNA, 2092 bp, synthetic construct
  source 1..2092: mol_type = other DNA
catggtgagcaagggcgaggagctgttcaccggggtggtgcccatcctggtcgagctggacggcgacgtaaacggccacaagttcagcgtgtccggcgagggcgagggcgatgccacctacggcaagctgaccctgaagttcatctgcaccaccggcaagctgcccgtgccctggcccaccctcgtgaccaccctgacctacggcgtgcagtgcttcagccgctaccccgaccacatgaagcagcacgacttcttcaagtccgccatgcccgaaggctacgtccaggagcgcaccatcttcttcaaggacgacggcaactacaagacccgcgccgaggtgaagttcgagggcgacaccctggtgaaccgcatcgagctgaagggcatcgacttcaaggaggacggcaacatcctggggcacaagctggagtacaactacaacagccacaacgtctatatcatggccgacaagcagaagaacggcatcaaggtgaacttcaagatccgccacaacatcgaggacggcagcgtgcagctcgccgaccactaccagcagaacacccccatcggcgacggccccgtgctgctgcccgacaaccactacctgagcacccagtccgccctgagcaaagaccccaacgagaagcgcgatcacatggtcctgctggagttcgtgaccgccgccgggatcactctcggcatggacgagctgtacaagtaaggatcctgcactagtgctgtcgactggtggactggtggactggtggactggtggactggtggactggtggactggtggactggtggactggtggactggtggacaagcttaaaaaaaaaaaaaaaaaaaaaaaaaaaaaaaaaaaaaaaaaaaaaaaaaaggaaaaaaaaaaaaaaaaaaaaaaaaaaaaaaaaaaaaaaaaggagaccgctagcctcgagttgacaattaaacattggcatagtatatctgcatagtataatacaactcactataggagggccatcatgtcaacagatgaaagaaaattggagatcatcagaaaagtgagttctgatattgatgagcctactctggaagcaattgaatatttgttatcaaccccttcagatatcccagaaccaatactgagagttattgaacaagcaatggcagaagaacctcttgaggaatacacttcagccaaagaggttattgagaaaagcagaacctaacaaagcccgccgaaaggcgggcttttttttgcggccgcctgtcagaccaagtttactcatatatactttagattgatttaaaacttcatttttaatttaaaaggatctaggtgaagatcctttttgataatctcatgaccaaaatcccttaacgtgagttttcgttccactgagcgtcagaccccgtagaaaagatcaaaggatcttcttgagatcctttttttctgcgcgtaatctgctgcttgcaaacaaaaaaaccaccgctaccagcggtggtttgtttgccggatcaagagctaccaactctttttccgaaggtaactggcttcagcagagcgcagataccaaatactgttcttctagtgtagccgtagttaggccaccacttcaagaactctgtagcaccgcctacatacctcgctctgctaatcctgttaccagtggctgctgccagtggcgataagtcgtgtcttaccgggttggactcaagacgatagttaccggataaggcgcagcggtcgggctgaacggggggttcgtgcacacagcccagcttggagcgaacgacctacaccgaactgagatacctacagcgtgagctatgagaaagcgccacgcttcccgaagggagaaaggcggacaggtatccggtaagcggcagggtcggaacaggagagcgcacgagggagcttccagggggaaacgcctggtatctttatagtcctgtcgggtttcgccacctctgacttgagcgtcgatttttgtgatgctcgtcaggggggcggagcctatggaaagacgtctaatacgactcactataagggaaataagagagaaaagaagagtaagaagaaatataagaccccggcgccgccac

SEQ ID NO: 47 - DNA, 1307 bp, synthetic construct
  source 1..1307: mol_type = other DNA
tcatacagaactggcgatcgttcggcgtatcgccaaaatcaccgccgtaagccgaccacgggttgccgttttcatcatatttaatcagcgactgatccacccagtcccagacgaagccgccctgtaaacggggatactgacgaaacgcctgccagtatttagcgaaaccgccaagactgttacccatcgcgtgggcgtattcgcaaaggatcagcgggcgcgtctctccaggtagcgaaagccattttttgatggaccatttcggcacagccgggaagggctggtcttcatccacgcgcgcgtacatcgggcaaataatatcggtggccgtggtgtcggctccgccgccttcatactgcaccgggcgggaaggatcgacagatttgatccagcgatacagcgcgtcgtgattagcgccgtggcctgattcattccccagcgaccagatgatcacactcgggtgattacgatcgcgctgcaccattcgcgttacgcgttcgctcatcgccggtagccagcgcggatcatcggtcagacgattcattggcaccatgccgtgggtttcaatattggcttcatccaccacatacaggccgtagcggtcgcacagcgtgtaccacagcggatggttcggataatgcgaacagcgcacggcgttaaagttgttctgcttcatcagcaggatatcctgcaccatcgtctgctcatccatgacctgaccatgcagaggatgatgctcgtgacggttaacgcctcgaatcagcaacggcttgccgttcagcagcagcagaccattttcaatccgcacctcgcggaaaccgacatcgcaggcttctgcttcaatcagcgtgccgtcggcggtgtgcagttcaaccaccgcacgatagagattcgggatttcggcgctccacagtttcgggttttcgacgttcagacgtagtgtgacgcgatcggcataaccaccacgctcatcgataatttcaccgccgaaaggcgcggtgccgctggcgacctgcgtttcaccctgccataaagaaactgttacccgtaggtagtcacgcaactcgccgcacatctgaacttcagcctccagtacagcgcggctgaaatcatcattaaagcgagtggcaacatggaaatcgctgatttgtgtagtcggtttatgcagcaacgagacgtcacggaaaatgccgctcatccgccacatatcctgatcttccagataactgccgtcactccagcgcagcaccatcaccgcgaggcggttttctccggcgcgtaaaaatgcgctcaggtcaaattcagac